European Patent Application EP 4 574 168 A1, published June 25, 2025. Title: Prime-Boost Immunization against influenza. Applicant: Unitectra AG. Application EP. The sequence listing filed with the application follows.

SEQUENCE LISTING (6 sequences)

SEQ ID NO: 1 - RNA, 11315 nt, synthetic construct
  source 1..11315: mol_type = other RNA; note = VSV HA
acgaagacaaacaaaccattattatcattaaaaggctcaggagaaactttaacagtaatcaaaatgtctgttacagtcaagagaatcattgacaacacagtcgtagttccaaaacttcctgcaaatgaggatccagtggaatacccggcagattacttcagaaaatcaaaggagattcctctttacatcaatactacaaaaagtttgtcagatctaagaggatatgtctaccaaggcctcaaatccggaaatgtatcaatcatacatgtcaacagctacttgtatggagcattaaaggacatccggggtaagttggataaagattggtcaagtttcggaataaacatcgggaaagcaggggatacaatcggaatatttgaccttgtatccttgaaagccctggacggcgtacttccagatggagtatcggatgcttccagaaccagcgcagatgacaaatggttgcctttgtatctacttggcttatacagagtgggcagaacacaaatgcctgaatacagaaaaaagctcatggatgggctgacaaatcaatgcaaaatgatcaatgaacagtttgaacctcttgtgccagaaggtcgtgacatttttgatgtgtggggaaatgacagtaattacacaaaaattgtcgctgcagtggacatgttcttccacatgttcaaaaaacatgaatgtgcctcgttcagatacggaactattgtttccagattcaaagattgtgctgcattggcaacatttggacacctctgcaaaataaccggaatgtctacagaagatgtaacgacctggatcttgaaccgagaagttgcagatgaaatggtccaaatgatgcttccaggccaagaaattgacaaggccgattcatacatgccttatttgatcgactttggattgtcttctaagtctccatattcttccgtcaaaaaccctgccttccacttctgggggcaattgacagctcttctgctcagatccaccagagcaaggaatgcccgacagcctgatgacattgagtatacatctcttactacagcaggtttgttgtacgcttatgcagtaggatcctctgccgacttggcacaacagttttgtgttggagataacaaatacactccagatgatagtaccggaggattgacgactaatgcaccgccacaaggcagagatgtggtcgaatggctcggatggtttgaagatcaaaacagaaaaccgactcctgatatgatgcagtatgcgaaaagagcagtcatgtcactgcaaggcctaagagagaagacaattggcaagtatgctaagtcagaatttgacaaatgaccctataattctcagatcacctattatatattatgctacatatgaaaaaaactaacagatatcatggataatctcacaaaagttcgtgagtatctcaagtcctattctcgtctggatcaggcggtaggagagatagatgagatcgaagcacaacgagctgaaaagtccaattatgagttgttccaagaggatggagtggaagagcatactaagccctcttattttcaggcagcagatgattctgacacagaatctgaaccagaaattgaagacaatcaaggcttgtatgcaccagatccagaagctgagcaagttgaaggctttatacaggggcctttagatgactatgcagatgaggaagtggatgttgtatttacttcggactggaaacagcctgagcttgaatctgacgagcatggaaagaccttacggttgacatcgccagagggtttaagtggagagcagaaatcccagtggctttcgacgattaaagcagtcgtgcaaagtgccaaatactggaatctggcagagtgcacatttgaagcatcgggagaaggggtcattatgaaggagcgccagataactccggatgtatataaggtcactccagtgatgaacacacatccgtcccaatcagaagcagtatcagatgtttggtctctctcaaagacatccatgactttccaacccaagaaagcaagtcttcagcctctcaccatatccttggatgaattgttctcatctagaggagagttcatctctgtcggaggtgacggacgaatgtctcataaagaggccatcctgctcggcctgagatacaaaaagttgtacaatcaggcgagagtcaaatattctctgtagactatgaaaaaaagtaacagatatcacgatctaagtgttatcccaatccattcatcatgagttccttaaagaagattctcggtctgaaggggaaaggtaagaaatctaagaaattagggatcgcaccacccccttatgaagaggacactagcatggagtatgctccgagcgctccaattgacaaatcctattttggagttgacgagatggacacctatgatccgaatcaattaagatatgagaaattcttctttacagtgaaaatgacggttagatctaatcgtccgttcagaacatactcagatgtggcagccgctgtatcccattgggatcacatgtacatcggaatggcagggaaacgtcccttctacaaaatcttggcttttttgggttcttctaatctaaaggccactccagcggtattggcagatcaaggtcaaccagagtatcacgctcactgcgaaggcagggcttatttgccacataggatggggaagacccctcccatgctcaatgtaccagagcacttcagaagaccattcaatataggtctttacaagggaacgattgagctcacaatgaccatctacgatgatgagtcactggaagcagctcctatgatctgggatcatttcaattcttccaaattttctgatttcagagagaaggccttaatgtttggcctgattgtcgagaaaaaggcatctggagcgtgggtcctggactctatcggccacttcaaatgagctagtctaacttctagcttctgaacaatccccggtttactcagtctcccctaattccagcctctcgaacaactaatatcctgtcttttctatccctatgaaaaaaactaacagagatcgatctgtttacgcgtaacatgaaggcaatactagtagttctgctatatacatttacaaccgcaaatgcagacacattatgtataggttatcatgcgaacaattcaacagacactgtagacacagtactagaaaagaatgtaacagtaacacactctgttaaccttctagaagacaagcataacgggaaactatgcaaactaagaggggtagccccattgcatttgggtaaatgtaacattgctggctggatcctgggaaatccagagtgtgaatcactctccacagcaagctcatggtcctacattgtggaaacatctagttcagacaatggaacgtgttacccaggagatttcatcgattatgaggagctaagagagcaattgagctcagtgtcatcatttgaaaggtttgagatattccccaagacaagttcatggcccaatcatgactcgaacaaaggtgtaacggcagcatgtcctcatgctggagcaaaaagcttctacaaaaatttaatatggctagttaaaaaaggaaattcatacccaaagctcagcaaatcctacattaatgataaagggaaagaagtcctcgtgctatggggcattcaccatccatctactagtgctgaccaacaaagtctctatcagaatgcagatgcatatgtttttgtggggtcatcaagatacagcaagaagttcaagccggaaatagcaataagacccaaagtgagggatcaagaagggagaatgaactattactggacactagtagagccgggagacaaaataacattcgaagcaactggaaatctagtggtaccgagatatgcattcgcaatggaaagaaatgctggatctggtattatcatttcagatacaccagtccacgattgcaatacaacttgtcagacacccaagggtgctataaacaccagcctcccatttcagaatatacatccgatcacaattggaaaatgtccaaaatatgtaaaaagcacaaaattgagactggccacaggattgaggaatgtcccgtctattcaatctagaggcctatttggggccattgccggtttcattgaaggggggtggacagggatggtagatggatggtacggttatcaccatcaaaatgagcaggggtcaggatatgcagccgacctgaagagcacacagaatgccattgacgagattactaacaaagtaaattctgttattgaaaagatgaatacacagttcacagcagtaggtaaagagttcaaccacctggaaaaaagaatagagaatttaaataaaaaagttgatgatggtttcctggacatttggacttacaatgccgaactgttggttctattggaaaatgaaagaactttggactaccacgattcaaatgtgaagaacttatatgaaaaggtaagaagccagctaaaaaacaatgccaaggaaattggaaacggctgctttgaattttaccacaaatgcgataacacgtgcatggaaagtgtcaaaaatgggacttatgactacccaaaatactcagaggaagcaaaattaaacagagaagaaatagatggggtaaagctggaatcaacaaggatttaccagattttggcgatctattcaactgtcgccagttcattggtactggtagtctccctgggggcaatcagtttctggatgtgctctaatgggtctctacagtgtagaatatgtatttaagctagccagattcttcatgtttggaccaaatcaacttgtgataccatgctcaaagaggcctcaattatatttgagtttttaatttttatgaaaaaaactaacagcaatcatggaagtccacgattttgagaccgacgagttcaatgatttcaatgaagatgactatgccacaagagaattcctgaatcccgatgagcgcatgacgtacttgaatcatgctgattacaacctgaattctcctctaattagtgatgatattgacaatttaatcaggaaattcaattctcttccaattccctcgatgtgggatagtaagaactgggatggagttcttgagatgttaacgtcatgtcaagccaatcccatcccaacatctcagatgcataaatggatgggaagttggttaatgtctgataatcatgatgccagtcaagggtatagttttttacatgaagtggacaaagaggcagaaataacatttgacgtggtggagaccttcatccgcggctggggcaacaaaccaattgaatacatcaaaaaggaaagatggactgactcattcaaaattctcgcttatttgtgtcaaaagtttttggacttacacaagttgacattaatcttaaatgctgtctctgaggtggaattgctcaacttggcgaggactttcaaaggcaaagtcagaagaagttctcatggaacgaacatatgcaggattagggttcccagcttgggtcctacttttatttcagaaggatgggcttacttcaagaaacttgatattctaatggaccgaaactttctgttaatggtcaaagatgtgattatagggaggatgcaaacggtgctatccatggtatgtagaatagacaacctgttctcagagcaagacatcttctcccttctaaatatctacagaattggagataaaattgtggagaggcagggaaatttttcttatgacttgattaaaatggtggaaccgatatgcaacttgaagctgatgaaattagcaagagaatcaaggcctttagtcccacaattccctcattttgaaaatcatatcaagacttctgttgatgaaggggcaaaaattgaccgaggtataagattcctccatgatcagataatgagtgtgaaaacagtggatctcacactggtgatttatggatcgttcagacattggggtcatccttttatagattattacactggactagaaaaattacattcccaagtaaccatgaagaaagatattgatgtgtcatatgcaaaagcacttgcaagtgatttagctcggattgttctatttcaacagttcaatgatcataaaaagtggttcgtgaatggagacttgctccctcatgatcatccctttaaaagtcatgttaaagaaaatacatggcccacagctgctcaagttcaagattttggagataaatggcatgaacttccgctgattaaatgttttgaaatacccgacttactagacccatcgataatatactctgacaaaagtcattcaatgaataggtcagaggtgttgaaacatgtccgaatgaatccgaacactcctatccctagtaaaaaggtgttgcagactatgttggacacaaaggctaccaattggaaagaatttcttaaagagattgatgagaagggcttagatgatgatgatctaattattggtcttaaaggaaaggagagggaactgaagttggcaggtagatttttctccctaatgtcttggaaattgcgagaatactttgtaattaccgaatatttgataaagactcatttcgtccctatgtttaaaggcctgacaatggcggacgatctaactgcagtcattaaaaagatgttagattcctcatccggccaaggattgaagtcatatgaggcaatttgcatagccaatcacattgattacgaaaaatggaataaccaccaaaggaagttatcaaacggcccagtgttccgagttatgggccagttcttaggttatccatccttaatcgagagaactcatgaattttttgagaaaagtcttatatactacaatggaagaccagacttgatgcgtgttcacaacaacacactgatcaattcaacctcccaacgagtttgttggcaaggacaagagggtggactggaaggtctacggcaaaaaggatggagtatcctcaatctactggttattcaaagagaggctaaaatcagaaacactgctgtcaaagtcttggcacaaggtgataatcaagttatttgcacacagtataaaacgaagaaatcgagaaacgttgtagaattacagggtgctctcaatcaaatggtttctaataatgagaaaattatgactgcaatcaaaatagggacagggaagttaggacttttgataaatgacgatgagactatgcaatctgcagattacttgaattatggaaaaataccgattttccgtggagtgattagagggttagagaccaagagatggtcacgagtgacttgtgtcaccaatgaccaaatacccacttgtgctaatataatgagctcagtttccacaaatgctctcaccgtagctcattttgctgagaacccaatcaatgccatgatacagtacaattattttgggacatttgctagactcttgttgatgatgcatgatcctgctcttcgtcaatcattgtatgaagttcaagataagataccgggcttgcacagttctactttcaaatacgccatgttgtatttggacccttccattggaggagtgtcgggcatgtctttgtccaggtttttgattagagccttcccagatcccgtaacagaaagtctctcattctggagattcatccatgtacatgctcgaagtgagcatctgaaggagatgagtgcagtatttggaaaccccgagatagccaagtttcgaataactcacatagacaagctagtagaagatccaacctctctgaacatcgctatgggaatgagtccagcgaacttgttaaagactgaggttaaaaaatgcttaatcgaatcaagacaaaccatcaggaaccaggtgattaaggatgcaaccatatatttgtatcatgaagaggatcggctcagaagtttcttatggtcaataaatcctctgttccctagatttttaagtgaattcaaatcaggcacttttttgggagtcgcagacgggctcatcagtctatttcaaaattctcgtactattcggaactcctttaagaaaaagtatcatagggaattggatgatttgattgtgaggagtgaggtatcctctttgacacatttagggaaacttcatttgagaaggggatcatgtaaaatgtggacatgttcagctactcatgctgacacattaagatacaaatcctggggccgtacagttattgggacaactgtaccccatccattagaaatgttgggtccacaacatcgaaaagagactccttgtgcaccatgtaacacatcagggttcaattatgtttctgtgcattgtccagacgggatccatgacgtctttagttcacggggaccattgcctgcttatctagggtctaaaacatctgaatctacatctattttgcagccttgggaaagggaaagcaaagtcccactgattaaaagagctacacgtcttagagatgctatctcttggtttgttgaacccgactctaaactagcaatgactatactttctaacatccactctttaacaggcgaagaatggaccaaaaggcagcatgggttcaaaagaacagggtctgcccttcataggttttcgacatctcggatgagccatggtgggttcgcatctcagagcactgcagcattgaccaggttgatggcaactacagacaccatgagggatctgggagatcagaatttcgactttttattccaagcaacgttgctctatgctcaaattaccaccactgttgcaagagacggatggatcaccagttgtacagatcattatcatattgcctgtaagtcctgtttgagacccatagaagagatcaccctggactcaagtatggactacacgcccccagatgtatcccatgtgctgaagacatggaggaatggggaaggttcgtggggacaagagataaaacagatctatcctttagaagggaattggaagaatttagcacctgctgagcaatcctatcaagtcggcagatgtataggttttctatatggagacttggcgtatagaaaatctactcatgccgaggacagttctctatttcctctatctatacaaggtcgtattagaggtcgaggtttcttaaaagggttgctagacggattaatgagagcaagttgctgccaagtaatacaccggagaagtctggctcatttgaagaggccggccaacgcagtgtacggaggtttgatttacttgattgataaattgagtgtatcacctccattcctttctcttactagatcaggacctattagagacgaattagaaacgattccccacaagatcccaacctcctatccgacaagcaaccgtgatatgggggtgattgtcagaaattacttcaaataccaatgccgtctaattgaaaagggaaaatacagatcacattattcacaattatggttattctcagatgtcttatccatagacttcattggaccattctctatttccaccaccctcttgcaaatcctatacaagccatttttatctgggaaagataagaatgagttgagagagctggcaaatctttcttcattgctaagatcaggagaggggtgggaagacatacatgtgaaattcttcaccaaggacatattattgtgtccagaggaaatcagacatgcttgcaagttcgggattgctaaggataataataaagacatgagctatcccccttggggaagggaatccagagggacaattacaacaatccctgtttattatacgaccaccccttacccaaagatgctagagatgcctccaagaatccaaaatcccctgctgtccggaatcaggttgggccaattaccaactggcgctcattataaaattcggagtatattacatggaatgggaatccattacagggacttcttgagttgtggagacggctccggagggatgactgctgcattactacgagaaaatgtgcatagcagaggaatattcaatagtctgttagaattatcagggtcagtcatgcgaggcgcctctcctgagccccccagtgccctagaaactttaggaggagataaatcgagatgtgtaaatggtgaaacatgttgggaatatccatctgacttatgtgacccaaggacttgggactatttcctccgactcaaagcaggcttggggcttcaaattgatttaattgtaatggatatggaagttcgggattcttctactagcctgaaaattgagacgaatgttagaaattatgtgcaccggattttggatgagcaaggagttttaatctacaagacttatggaacatatatttgtgagagcgaaaagaatgcagtaacaatccttggtcccatgttcaagacggtcgacttagttcaaacagaatttagtagttctcaaacgtctgaagtatatatggtatgtaaaggtttgaagaaattaatcgatgaacccaatcccgattggtcttccatcaatgaatcctggaaaaacctgtacgcattccagtcatcagaacaggaatttgccagagcaaagaaggttagtacatactttaccttgacaggtattccctcccaattcattcctgatccttttgtaaacattgagactatgctacaaatattcggagtacccacgggtgtgtctcatgcggctgccttaaaatcatctgatagacctgcagatttattgaccattagccttttttatatggcgattatatcgtattataacatcaatcatatcagagtaggaccgatacctccgaaccccccatcagatggaattgcacaaaatgtggggatcgctataactggtataagcttttggctgagtttgatggagaaagacattccactatatcaacagtgtttagcagttatccagcaatcattcccgattaggtgggaggctgtttcagtaaaaggaggatacaagcagaagtggagtactagaggtgatgggctcccaaaagatacccgaatttcagactccttggccccaatcgggaactggatcagatctctggaattggtccgaaaccaagttcgtctaaatccattcaatgagatcttgttcaatcagctatgtcgtacagtggataatcatttgaaatggtcaaatttgcgaagaaacacaggaatgattgaatggatcaatagacgaatttcaaaagaagaccggtctatactgatgttgaagagtgacctacacgaggaaaactcttggagagattaaaaaatcatgaggagactccaaactttaagtatgaaaaaaactttgatccttaagaccctcttgtggtttttattttttatctggttttgtggtcttcgt

SEQ ID NO: 2 - RNA, 13554 nt, synthetic construct
  source 1..13554: mol_type = other RNA; note = NS1(1-126)
agcgaaagcaggtcaaatatattcaatatggagagaataaaagaactgagagatctaatgtcgcagtcccgcactcgcgagatactcactaagaccactgtggaccatatggccataatcaaaaagtacacatcaggaaggcaagagaagaaccccgcactcagaatgaagtggatgatggcaatgagatacccaattacagcagacaagagaataatggacatgattccagagaggaatgaacaaggacaaaccctctggagcaaaacaaacgatgctggatcagaccgagtgatggtatcacctctggccgtaacatggtggaataggaatggcccaacaacaagtacagttcattaccctaaggtatataaaacttatttcgaaaaggtcgaaaggttgaaacatggtaccttcggccctgtccacttcagaaatcaagttaaaataaggaggagagttgatacaaaccctggccatgcagatctcagtgccaaggaggcacaggatgtgattatggaagttgttttcccaaatgaagtgggggcaagaatactgacatcagagtcacagctggcaataacaaaagagaagaaagaagagctccaggattgtaaaattgctcccttgatggtggcgtacatgctagaaagagaattggtccgtaaaacaaggtttctcccagtagccggcggaacaggcagtgtttatattgaagtgttgcacttaacccaagggacgtgctgggagcagatgtacactccaggaggagaagtgagaaatgatgatgttgaccaaagtttgattatcgctgctagaaacatagtaagaagagcagcagtgtcagcagacccattagcatctctcttggaaatgtgccacagcacacagattggaggagtaaggatggtggacatccttagacagaatccaactgaggaacaagccgtagacatatgcaaggcagcaatagggttgaggattagctcatctttcagttttggtgggttcactttcaaaaggacaagcggatcatcagtcaagaaagaagaagaagtgctaacgggcaacctccaaacactgaaaataagagtacatgaagggtatgaagaattcacaatggttgggagaagagcaacagctattctcagaaaggcaaccaggagattgatccagttgatagtaagcgggagagacgagcagtcaattgctgaggcaataattgtggccatggtattctcacaagaggattgcatgatcaaggcagttaggggcgatctgaactttgtcaatagggcaaaccagcgactgaaccccatgcaccaactcttgaggcatttccaaaaagatgcaaaagtgcttttccagaactggggaattgaatccatcgacaatgtgatgggaatgatcggaatactgcccgacatgaccccaagcacggagatgtcgctgagagggataagagtcagcaaaatgggagtagatgaatactccagcacggagagagtggtagtgagtattgaccgatttttaagggttagagatcaaagagggaacgtactattgtctcccgaagaagtcagtgaaacgcaaggaactgagaggttgacaataacttattcgtcatcaatgatgtgggagatcaatggccctgagtcagtgctagtcaacacttatcaatggataatcaggaactgggaaattgtgaaaattcaatggtcacaagatcccacaatgttatacaacaaaatggaatttgaaccatttcagtctcttgtccctaaggcaaccagaagccggtacagtggattcgtaaggacactgttccagcaaatgcgggatgtgcttgggacatttgacactgtccaaataataaaacttctcccctttgctgctgctccaccagaacagagtaggatgcaattttcctcattgactgtgaatgtgagaggatcagggttgaggatactggtaagaggcaattctccagtattcaattacaacaaggcaaccaaacgacttacagttcttggaaaggatgcaggtgcattgactgaagatccagatgaaggcacatctggggtggagtctgctgtcctgagaggatttctcattttgggcaaagaagacaagagatatggcccagcattaagcatcaatgaactgagcaatcttgcaaaaggagagaaggctaatgtgctaattgggcaaggggacgtagtgttggtaatgaaacgaaaacgggactctagcatacttactgacagccagacagcgaccaaaagaattcggatggccatcaattagtgtcgaattgtttaaaaacgaccttgtttctactagcgaaagcaggcaaaccatttgaatggatgtcaatccgactctacttttcctaaaaattccagcgcaaaatgccataagcaccacattcccttatactggagatcctccatacagccatggaacaggaacaggatacaccatggacacagtaaacagaacacaccaatactcagaaaagggaaagtggacgacaaacacagagactggtgcaccccagctcaacccgattgatggaccactacctgaggataatgaaccaagtgggtatgcacaaacagactgtgttctagaggctatggctttccttgaagaatcccacccaggaatatttgagaattcatgccttgaaacaatggaagttgttcaacaaacaagggtagataaactaactcaaggtcgccagacttatgattggacattaaacagaaatcaaccggcagcaactgcattggccaacaccatagaagtctttagatcgaatggcctaacagctaatgagtcaggaaggctaatagatttcttaaaggatgtaatggaatcaatgaacaaagaggaaatagagataacaacccactttcaaagaaaaaggagagtaagagacaacatgaccaagaagatggtcacgcaaagaacaatagggaagaaaaaacaaagactgaataagagaggctatctaataagagcactgacattaaatacgatgaccaaagatgcagagagaggcaagttaaaaagaagggctatcgcaacacctgggatgcagattagaggtttcgtatactttgttgaaactttagctaggagcatttgcgaaaagcttgaacagtctgggctcccagtagggggcaatgaaaagaaggccaaactggcaaatgttgtgagaaagatgatgactaattcacaagacacagagatttctttcacaatcactggggacaacactaagtggaatgaaaatcaaaatcctcgagtgttcctggcgatgattacatatatcaccagaaatcaacccgagtggttcagaaacatcctgagcatggcacccataatgttctcaaacaaaatggcaagactagggaaagggtacatgttcgagagtaaaagaatgaagattcgaacacaaataccagcagaaatgctagcaagcattgacctgaagtacttcaatgaatcaacaaagaagaaaattgagaaaataaggcctcttctaatagatggcacagcatcactgagtcctgggatgatgatgggcatgttcaacatgctaagtacggtcttgggagtctcgatactgaatcttggacaaaagaaatacaccaagacaatatactggtgggatgggctccaatcatccgacgattttgctctcatagtgaatgcaccaaaccatgagggaatacaagcaggagtggacagattctacaggacctgcaagttagtgggaatcaacatgagcaaaaagaagtcctatataaataagacagggacatttgaattcacaagctttttttatcgctatggatttgtggctaattttagcatggagctacccagctttggagtgtctggagtaaatgaatcagctgacatgagtattggagtaacagtgataaagaacaacatgataaacaatgaccttggacctgcaacggcccagatggctcttcaattgttcatcaaagactacagatacacatataggtgccataggggagacacacaaattcagacgagaagatcatttgagttaaagaagctgtgggatcaaacccaatcaaaggtagggctattagtatcagatggaggaccaaacttatacaatatacggaatcttcacattcctgaagtctgcttaaaatgggagctaatggatgatgattatcggggaagactttgtaatcccctgaatccctttgtcagtcataaagagattgattctgtaaacaatgctgtggtaatgccagcccatggtccagccaaaagcatggaatatgatgccgttgcaactacacattcctggattcccaagaggaatcgttctattctcaacacaagccaaaggggaattcttgaggatgaacagatgtaccagaagtgctgcaatctattcgagaaatttttccctagcagttcatataggagaccggttggaatttctagcatggtggaggccatggtgtctagggcccggattgatgccagggtcgacttcgagtctggacggatcaagaaagaagagttctctgagatcatgaagatctgttccaccattgaagaactcagacggcaaaaataatgaatttagcttgtccttcatgaaaaaatgccttgtttctactagcaaaagcaggtactgatccaaaatggaagactttgtgcgacaatgcttcaatccaatgatcgtcgagcttgcggaaaaggcaatgaaagaatatggggaagatccgaaaatcgaaactaacaagtttgctgcaatatgcacacatttggaagtttgtttcatgtattcggatttccatttcatcgacgaacggggtgaatcaataattgtagaatctggtgacccgaatgcactattgaagcaccgatttgagataattgaaggaagagaccgaatcatggcctggacagtggtgaacagtatatgtaacacaacaggggtagagaagcctaaatttcttcctgatttgtatgattacaaagagaaccggttcattgaaattggagtaacacggagggaagtccacatatattacctagagaaagccaacaaaataaaatctgagaagacacacattcacatcttttcattcactggagaggagatggccaccaaagcggactacacccttgacgaagagagcagggcaagaatcaaaactaggcttttcactataagacaagaaatggccagtaggagtctatgggattcctttcgtcagtccgaaagaggcgaagagacaattgaagaaaaatttgagattacaggaactatgcgcaagcttgccgaccaaagtctcccaccgaacttctccagccttgaaaactttagagcctatgtagatggattcgagccgaacggctgcattgagggcaagctttcccaaatgtcaaaagaagtgaacgccaaaattgaaccattcttgaggacgacaccacgccccctcagattgcctgatgggcctctttgccatcagcggtcaaagttcctgctgatggatgctctgaaattaagtattgaagacccgagtcacgagggggagggaataccactatatgatgcaatcaaatgcatgaagacattctttggctggaaagagcctaacatagtcaaaccacatgagaaaggcataaatcccaattacctcatggcttggaagcaggtgctagcagagctacaggacattgaaaatgaagagaagatcccaaggacaaagaacatgaagagaacaagccaattgaagtgggcactcggtgaaaatatggcaccagaaaaagtagactttgatgactgcaaagatgttggagaccttaaacagtatgacagtgatgagccagagcccagatctctagcaagctgggtccaaaatgaattcaataaggcatgtgaattgactgattcaagctggatagaacttgatgaaataggagaagatgttgccccgattgaacatatcgcaagcatgaggaggaactattttacagcagaagtgtcccactgcagggctactgaatacataatgaagggagtgtacataaatacggccttgctcaatgcatcctgtgcagccatggatgactttcagctgatcccaatgataagcaaatgtaggaccaaagaaggaagacggaaaacaaacctgtatgggttcattataaaaggaaggtctcatttgagaaatgatactgatgtggtgaactttgtaagtatggagttctcactcactgacccgagactggagccacacaaatgggaaaaatactgtgttcttgaaataggagacatgctcttgaggactgcgataggccaagtgtcgaggcccatgttcctatatgtgagaaccaatggaacctccaagatcaagatgaaatggggcatggaactgaggcgctgccttcttcagtctcttcagcagattgagagcatgattgaggccgagtcttctgtcaaagagaaagacatgaccaaggaattctttgaaaacaaatcggaaacatggccaatcggagagtcacccaggggagtggaggaaggctctattgggaaagtgtgcaggaccttactggcaaaatctgtattcaacagtctatatgcgtctccacaacttgaggggttttcggctgaatcgagaaaattgcttctcattgttcaggcacttagggacaacctggaacctggaaccttcgatcttggggggctatatgaagcaatcgaggagtgcctgattaatgatccctgggttttgcttaatgcatcttggttcaactccttcctcacacatgcactgaagtagttgtggcaatgctactatttgctatccatactgtccaaaaaagtaccttgtttctactagcaaaagcaggggaaaacaaaagcaacaaaaatgaaggcaatactagtagttctgctatatacatttacaaccgcaaatgcagacacattatgtataggttatcatgcgaacaattcaacagacactgtagacacagtactagaaaagaatgtaacagtaacacactctgttaaccttctagaagacaagcataacgggaaactatgcaaactaagaggggtagccccattgcatttgggtaaatgtaacattgctggctggatcctgggaaatccagagtgtgaatcactctccacagcaagctcatggtcctacattgtggaaacatctagttcagacaatggaacgtgttacccaggagatttcatcgattatgaggagctaagagagcaattgagctcagtgtcatcatttgaaaggtttgagatattccccaagacaagttcatggcccaatcatgactcgaacaaaggtgtaacggcagcatgtcctcatgctggagcaaaaagcttctacaaaaatttaatatggctagttaaaaaaggaaattcatacccaaagctcagcaaatcctacattaatgataaagggaaagaagtcctcgtgctatggggcattcaccatccatctactagtgctgaccaacaaagtctctatcagaatgcagatgcatatgtttttgtggggtcatcaagatacagcaagaagttcaagccggaaatagcaataagacccaaagtgagggatcaagaagggagaatgaactattactggacactagtagagccgggagacaaaataacattcgaagcaactggaaatctagtggtaccgagatatgcattcgcaatggaaagaaatgctggatctggtattatcatttcagatacaccagtccacgattgcaatacaacttgtcagacacccaagggtgctataaacaccagcctcccatttcagaatatacatccgatcacaattggaaaatgtccaaaatatgtaaaaagcacaaaattgagactggccacaggattgaggaatgtcccgtctattcaatctagaggcctatttggggccattgccggtttcattgaaggggggtggacagggatggtagatggatggtacggttatcaccatcaaaatgagcaggggtcaggatatgcagccgacctgaagagcacacagaatgccattgacgagattactaacaaagtaaattctgttattgaaaagatgaatacacagttcacagcagtaggtaaagagttcaaccacctggaaaaaagaatagagaatttaaataaaaaagttgatgatggtttcctggacatttggacttacaatgccgaactgttggttctattggaaaatgaaagaactttggactaccacgattcaaatgtgaagaacttatatgaaaaggtaagaagccagctaaaaaacaatgccaaggaaattggaaacggctgctttgaattttaccacaaatgcgataacacgtgcatggaaagtgtcaaaaatgggacttatgactacccaaaatactcagaggaagcaaaattaaacagagaagaaatagatggggtaaagctggaatcaacaaggatttaccagattttggcgatctattcaactgtcgccagttcattggtactggtagtctccctgggggcaatcagtttctggatgtgctctaatgggtctctacagtgtagaatatgtatttaacattaggatttcagaagcatgagaaaaacacccttgtttctactagcaaaagcagggtagataatcactcaatggcgtctcaaggcaccaaacgatcatatgaacaaatggagactggtggggagcgccaggatgccacagaaatcagagcatctgtcggaagaatgattggtggaatcgggagattctacatccaaatgtgcactgaactcaaactcagtgattatgatggacgactaatccagaatagcataacaatagagaggatggtgctttctgcttttgatgagagaagaaataaatacctagaagagcatcccagtgctgggaaggaccccaagaaaacaggaggacccatatatagaagagtagacggaaagtggatgagagaactcatcctttatgacaaagaagaaataaggagagtttggcgccaagcaaacaatggcgaagatgcaacagcaggtattactcatatcatgatttggcattccaacctgaatgatgccacatatcagagaacaagagcgcttgttcgcaccggaatggatcccagaatgtgctctctaatgcaaggttcaacacttcccagaaggtctggtgccgcaggtgctgcggtgaaaggagttggaacaatagcaatggagttaatcagaatgatcaaacgtggaatcaatgaccgaaatttctggaggggtgaaaatggacgaaggacaagggttgcttatgaaagaatgtgcaatatcctcaaaggaaaatttcaaacagctgcccagagggcaatgatggatcaagtaagagaaagtcgaaacccaggaaacgctgagattgaagacctcattttcctggcacggtcagcactcattctgaggggatcagttgcacataaatcctgcctgcctgcttgtgtgtatgggcttgcagtagcaagtgggcatgactttgaaagggaagggtactcactggtcgggatagacccattcaaattactccaaaacagccaagtggtcagcctgatgagaccaaatgaaaacccagctcacaagagtcaattggtgtggatggcatgccactctgctgcatttgaagatttaagagtatcaagtttcataagaggaaagaaagtgattccaagaggaaagctttccacaagaggggtccagattgcttcaaatgagaatgtggaaatcatggactccaataccctggaactgagaagcagatactgggccataaggaccaggagtggaggaaataccaatcaacaaaaggcatccgcaggccagatcagtgtgcagcctacattctcagtgcagcggaatctcccttttgaaagagcaaccgttatggcagcattcagcgggaacaatgaaggacggacatccgacatgcgaacagaagttataagaatgatggaaagtgcaaagccagaagatttgtccttccaggggcggggagtcttcgagctctcggacgaaaaggcaacgaacccgatcgtgccttcctttgacatgagtaatgaagggtcttatttcttcggagacaatgcagaggagtatgacagttgaggaaaaatacccttgtttctactagcaaaagcaggagtttaaaatgaatccaaaccaaaagataataaccattggttcggtctgtatgacaattggaatggctaacttaatattacaaattggaaacataatctcaacatggattagccactcaattcaacttgggaatcaaaatcagattgaaacatgcaatcaaagcgtcattacttatgaaaacaacacttgggtaaatcagacatatgttaacatcagcaacaccaactttgctgctggacagtcagtggtttccgtgaaattagcgggcaattcctctctctgccctgttagtggatgggctatatacagtaaagacaacagcgtaagaatcggttccaagggggatgtgtttgtcataagggaaccattcatatcatgctcccccttggaatgcagaaccttcttcttgactcaaggggccttgctaaatgacaaacattccaatggaaccattaaagacaggagcccatatcgaaccctaatgagctgtcctattggtgaagttccctctccatacaactcaagatttgagtcagtcgcttggtcagcaagtgcttgtcatgatggcatcaattggctaacaattggaatttctggcccagacaatggggcagtggctgtgttaaagtacaacggcataataacagacactatcaagagttggagaaacaatatattgagaacacaagagtctgaatgtgcatgtgtaaatggttcttgctttactgtaatgaccgatggaccaagtaatggacaggcctcatacaagatcttcagaatagaaaagggaaaaatagtcaaatcagtcgaaatgaatgcccctaattatcactatgaggaatgctcctgttatcctgattctagtgaaatcacatgtgtgtgcagggataactggcatggctcgaatcgaccgtgggtgtctttcaaccagaatctggaatatcagataggatacatatgcagtgggattttcggagacaatccacgccctaatgataagacaggcagttgtggtccagtatcgtctaatggagcaaatggagtaaaaggattttcattcaaatacggcaatggtgtttggatagggagaactaaaagcattagttcaagaaacggttttgagatgatttgggatccgaacggatggactgggacagacaataacttctcaataaagcaagatatcgtaggaataaatgagtggtcaggatatagcgggagttttgttcagcatccagaactaacagggctggattgtataagaccttgcttctgggttgaactaatcagagggcgacccaaagagaacacaatctggactagcgggagcagcatatccttttgtggtgtaaacagtgacactgtgggttggtcttggccagacggtgctgagttgccatttaccattgacaagtaatttgttcaaaaaactccttgtttctactagcaaaagcaggtagatatttaaagatgagtcttctaaccgaggtcgaaacgtacgttctttctatcatcccgtcaggccccctcaaagccgagatcgcgcagagactggaaagtgtctttgcaggaaagaacacagatcttgaggctctcatggaatggctaaagacaagaccaatcttgtcacctctgactaagggaattttaggatttgtgttcacgctcaccgtgcccagtgagcgaggactgcagcgtagacgctttgtccaaaatgccctaaatgggaatggggacccgaacaacatggatagagcagttaaactatacaagaagctcaaaagagaaataacgttccatggggccaaggaggtgtcactaagctattcaactggtgcacttgccagttgcatgggcctcatatacaacaggatgggaacagtgaccacagaagctgcttttggtctagtgtgtgccacttgtgaacagattgctgattcacagcatcggtctcacagacagatggctactaccaccaatccactaatcaggcatgaaaacagaatggtgctggctagcactacggcaaaggctatggaacagatggctggatcgagtgaacaggcagcggaggccatggaggttgctaatcagactaggcagatggtacatgcaatgagaactattgggactcatcctagctccagtgctggtctgaaagatgaccttcttgaaaatttgcaggcctaccagaagcgaatgggagtgcagatgcagcgattcaagtgatcctctcgtcattgcagcaaatatcattgggatcttgcacctgatattgtggattactgatcgtctttttttcaaatgtatttatcgtcgctttaaatacggtttgaaaagagggccttctacggaaggagtgcctgagtccatgagggaagaatatcaacaggaacagcagagtgctgtggatgttgacgatggtcattttgtcaacatagagctggagtaaaaaactaccttgtttctactagcaaaagcagggtgacaaaaacataatggactccaacaccatgtcaagctttcaggtagactgtttcctttggcatatccgcaagcgatttgcagacaatggattgggtgatgccccattccttgatcggctccgccgagatcaaaagtccttaaaaggaagaggcaacacccttggcctcgatatcgaaacagccactcttgttgggaaacaaatcgtggaatggatcttgaaagaggaatccagcgagacacttagaatgacaattgcatctgtacctacttcgcgctacctttctgacatgaccctcgaggaaatgtcacgagactggttcatgctcatgcctaggcaaaagataataggccctctttgcgtgcgattggaccaggcgatcatggaaaagtagatcttgattaattaagagggagcaatagttggagaaatttcaccattaccttctcttccaggacatacttatgaggatgtcaaaaatgcagttggggtcctcatcggaggacttgaatggaatggtaacacggttcgagtctctgaaaatatacagagattcgcttggagaaactgtgatgagaatgggagaccttcactacctccagagcagaaatgaaaagtggcgagagcaattgggacagaaatttgaggaaataaggtggttaattgaagaaatgcggcacagattgaaagcgacagagaatagtttcgaacaaataacatttatgcaagccttacaactattgcttgaagtagaacaagagataagagctttctcgtttcagcttatttaatgataaaaaacacccttgtttctact

SEQ ID NO: 3 - RNA, 13554 nt, synthetic construct
  source 1..13554: mol_type = other RNA; note = NS1(1-126)-deltaPAX
agcgaaagcaggtcaaatatattcaatatggagagaataaaagaactgagagatctaatgtcgcagtcccgcactcgcgagatactcactaagaccactgtggaccatatggccataatcaaaaagtacacatcaggaaggcaagagaagaaccccgcactcagaatgaagtggatgatggcaatgagatacccaattacagcagacaagagaataatggacatgattccagagaggaatgaacaaggacaaaccctctggagcaaaacaaacgatgctggatcagaccgagtgatggtatcacctctggccgtaacatggtggaataggaatggcccaacaacaagtacagttcattaccctaaggtatataaaacttatttcgaaaaggtcgaaaggttgaaacatggtaccttcggccctgtccacttcagaaatcaagttaaaataaggaggagagttgatacaaaccctggccatgcagatctcagtgccaaggaggcacaggatgtgattatggaagttgttttcccaaatgaagtgggggcaagaatactgacatcagagtcacagctggcaataacaaaagagaagaaagaagagctccaggattgtaaaattgctcccttgatggtggcgtacatgctagaaagagaattggtccgtaaaacaaggtttctcccagtagccggcggaacaggcagtgtttatattgaagtgttgcacttaacccaagggacgtgctgggagcagatgtacactccaggaggagaagtgagaaatgatgatgttgaccaaagtttgattatcgctgctagaaacatagtaagaagagcagcagtgtcagcagacccattagcatctctcttggaaatgtgccacagcacacagattggaggagtaaggatggtggacatccttagacagaatccaactgaggaacaagccgtagacatatgcaaggcagcaatagggttgaggattagctcatctttcagttttggtgggttcactttcaaaaggacaagcggatcatcagtcaagaaagaagaagaagtgctaacgggcaacctccaaacactgaaaataagagtacatgaagggtatgaagaattcacaatggttgggagaagagcaacagctattctcagaaaggcaaccaggagattgatccagttgatagtaagcgggagagacgagcagtcaattgctgaggcaataattgtggccatggtattctcacaagaggattgcatgatcaaggcagttaggggcgatctgaactttgtcaatagggcaaaccagcgactgaaccccatgcaccaactcttgaggcatttccaaaaagatgcaaaagtgcttttccagaactggggaattgaatccatcgacaatgtgatgggaatgatcggaatactgcccgacatgaccccaagcacggagatgtcgctgagagggataagagtcagcaaaatgggagtagatgaatactccagcacggagagagtggtagtgagtattgaccgatttttaagggttagagatcaaagagggaacgtactattgtctcccgaagaagtcagtgaaacgcaaggaactgagaggttgacaataacttattcgtcatcaatgatgtgggagatcaatggccctgagtcagtgctagtcaacacttatcaatggataatcaggaactgggaaattgtgaaaattcaatggtcacaagatcccacaatgttatacaacaaaatggaatttgaaccatttcagtctcttgtccctaaggcaaccagaagccggtacagtggattcgtaaggacactgttccagcaaatgcgggatgtgcttgggacatttgacactgtccaaataataaaacttctcccctttgctgctgctccaccagaacagagtaggatgcaattttcctcattgactgtgaatgtgagaggatcagggttgaggatactggtaagaggcaattctccagtattcaattacaacaaggcaaccaaacgacttacagttcttggaaaggatgcaggtgcattgactgaagatccagatgaaggcacatctggggtggagtctgctgtcctgagaggatttctcattttgggcaaagaagacaagagatatggcccagcattaagcatcaatgaactgagcaatcttgcaaaaggagagaaggctaatgtgctaattgggcaaggggacgtagtgttggtaatgaaacgaaaacgggactctagcatacttactgacagccagacagcgaccaaaagaattcggatggccatcaattagtgtcgaattgtttaaaaacgaccttgtttctactagcgaaagcaggcaaaccatttgaatggatgtcaatccgactctacttttcctaaaaattccagcgcaaaatgccataagcaccacattcccttatactggagatcctccatacagccatggaacaggaacaggatacaccatggacacagtaaacagaacacaccaatactcagaaaagggaaagtggacgacaaacacagagactggtgcaccccagctcaacccgattgatggaccactacctgaggataatgaaccaagtgggtatgcacaaacagactgtgttctagaggctatggctttccttgaagaatcccacccaggaatatttgagaattcatgccttgaaacaatggaagttgttcaacaaacaagggtagataaactaactcaaggtcgccagacttatgattggacattaaacagaaatcaaccggcagcaactgcattggccaacaccatagaagtctttagatcgaatggcctaacagctaatgagtcaggaaggctaatagatttcttaaaggatgtaatggaatcaatgaacaaagaggaaatagagataacaacccactttcaaagaaaaaggagagtaagagacaacatgaccaagaagatggtcacgcaaagaacaatagggaagaaaaaacaaagactgaataagagaggctatctaataagagcactgacattaaatacgatgaccaaagatgcagagagaggcaagttaaaaagaagggctatcgcaacacctgggatgcagattagaggtttcgtatactttgttgaaactttagctaggagcatttgcgaaaagcttgaacagtctgggctcccagtagggggcaatgaaaagaaggccaaactggcaaatgttgtgagaaagatgatgactaattcacaagacacagagatttctttcacaatcactggggacaacactaagtggaatgaaaatcaaaatcctcgagtgttcctggcgatgattacatatatcaccagaaatcaacccgagtggttcagaaacatcctgagcatggcacccataatgttctcaaacaaaatggcaagactagggaaagggtacatgttcgagagtaaaagaatgaagattcgaacacaaataccagcagaaatgctagcaagcattgacctgaagtacttcaatgaatcaacaaagaagaaaattgagaaaataaggcctcttctaatagatggcacagcatcactgagtcctgggatgatgatgggcatgttcaacatgctaagtacggtcttgggagtctcgatactgaatcttggacaaaagaaatacaccaagacaatatactggtgggatgggctccaatcatccgacgattttgctctcatagtgaatgcaccaaaccatgagggaatacaagcaggagtggacagattctacaggacctgcaagttagtgggaatcaacatgagcaaaaagaagtcctatataaataagacagggacatttgaattcacaagctttttttatcgctatggatttgtggctaattttagcatggagctacccagctttggagtgtctggagtaaatgaatcagctgacatgagtattggagtaacagtgataaagaacaacatgataaacaatgaccttggacctgcaacggcccagatggctcttcaattgttcatcaaagactacagatacacatataggtgccataggggagacacacaaattcagacgagaagatcatttgagttaaagaagctgtgggatcaaacccaatcaaaggtagggctattagtatcagatggaggaccaaacttatacaatatacggaatcttcacattcctgaagtctgcttaaaatgggagctaatggatgatgattatcggggaagactttgtaatcccctgaatccctttgtcagtcataaagagattgattctgtaaacaatgctgtggtaatgccagcccatggtccagccaaaagcatggaatatgatgccgttgcaactacacattcctggattcccaagaggaatcgttctattctcaacacaagccaaaggggaattcttgaggatgaacagatgtaccagaagtgctgcaatctattcgagaaatttttccctagcagttcatataggagaccggttggaatttctagcatggtggaggccatggtgtctagggcccggattgatgccagggtcgacttcgagtctggacggatcaagaaagaagagttctctgagatcatgaagatctgttccaccattgaagaactcagacggcaaaaataatgaatttagcttgtccttcatgaaaaaatgccttgtttctactagcaaaagcaggtactgatccaaaatggaagactttgtgcgacaatgcttcaatccaatgatcgtcgagcttgcggaaaaggcaatgaaagaatatggggaagatccgaaaatcgaaactaacaagtttgctgcaatatgcacacatttggaagtttgtttcatgtattcggatttccatttcatcgacgaacggggtgaatcaataattgtagaatctggtgacccgaatgcactattgaagcaccgatttgagataattgaaggaagagaccgaatcatggcctggacagtggtgaacagtatatgtaacacaacaggggtagagaagcctaaatttcttcctgatttgtatgattacaaagagaaccggttcattgaaattggagtaacacggagggaagtccacatatattacctagagaaagccaacaaaataaaatctgagaagacacacattcacatcttttcattcactggagaggagatggccaccaaagcggactacacccttgacgaagagagcagggcaagaatcaaaactaggcttttcactataagacaagaaatggccagtaggagtctatgggattcgttcagacagtccgaaagaggcgaagagacaattgaagaaaaatttgagattacaggaactatgcgcaagcttgccgaccaaagtctcccaccgaacttctccagccttgaaaactttagagcctatgtagatggattcgagccgaacggctgcattgagggcaagctttcccaaatgtcaaaagaagtgaacgccaaaattgaaccattcttgaggacgacaccacgccccctcagattgcctgatgggcctctttgccatcagcggtcaaagttcctgctgatggatgctctgaaattaagtattgaagacccgagtcacgagggggagggaataccactatatgatgcaatcaaatgcatgaagacattctttggctggaaagagcctaacatagtcaaaccacatgagaaaggcataaatcccaattacctcatggcttggaagcaggtgctagcagagctacaggacattgaaaatgaagagaagatcccaaggacaaagaacatgaagagaacaagccaattgaagtgggcactcggtgaaaatatggcaccagaaaaagtagactttgatgactgcaaagatgttggagaccttaaacagtatgacagtgatgagccagagcccagatctctagcaagctgggtccaaaatgaattcaataaggcatgtgaattgactgattcaagctggatagaacttgatgaaataggagaagatgttgccccgattgaacatatcgcaagcatgaggaggaactattttacagcagaagtgtcccactgcagggctactgaatacataatgaagggagtgtacataaatacggccttgctcaatgcatcctgtgcagccatggatgactttcagctgatcccaatgataagcaaatgtaggaccaaagaaggaagacggaaaacaaacctgtatgggttcattataaaaggaaggtctcatttgagaaatgatactgatgtggtgaactttgtaagtatggagttctcactcactgacccgagactggagccacacaaatgggaaaaatactgtgttcttgaaataggagacatgctcttgaggactgcgataggccaagtgtcgaggcccatgttcctatatgtgagaaccaatggaacctccaagatcaagatgaaatggggcatggaactgaggcgctgccttcttcagtctcttcagcagattgagagcatgattgaggccgagtcttctgtcaaagagaaagacatgaccaaggaattctttgaaaacaaatcggaaacatggccaatcggagagtcacccaggggagtggaggaaggctctattgggaaagtgtgcaggaccttactggcaaaatctgtattcaacagtctatatgcgtctccacaacttgaggggttttcggctgaatcgagaaaattgcttctcattgttcaggcacttagggacaacctggaacctggaaccttcgatcttggggggctatatgaagcaatcgaggagtgcctgattaatgatccctgggttttgcttaatgcatcttggttcaactccttcctcacacatgcactgaagtagttgtggcaatgctactatttgctatccatactgtccaaaaaagtaccttgtttctactagcaaaagcaggggaaaacaaaagcaacaaaaatgaaggcaatactagtagttctgctatatacatttacaaccgcaaatgcagacacattatgtataggttatcatgcgaacaattcaacagacactgtagacacagtactagaaaagaatgtaacagtaacacactctgttaaccttctagaagacaagcataacgggaaactatgcaaactaagaggggtagccccattgcatttgggtaaatgtaacattgctggctggatcctgggaaatccagagtgtgaatcactctccacagcaagctcatggtcctacattgtggaaacatctagttcagacaatggaacgtgttacccaggagatttcatcgattatgaggagctaagagagcaattgagctcagtgtcatcatttgaaaggtttgagatattccccaagacaagttcatggcccaatcatgactcgaacaaaggtgtaacggcagcatgtcctcatgctggagcaaaaagcttctacaaaaatttaatatggctagttaaaaaaggaaattcatacccaaagctcagcaaatcctacattaatgataaagggaaagaagtcctcgtgctatggggcattcaccatccatctactagtgctgaccaacaaagtctctatcagaatgcagatgcatatgtttttgtggggtcatcaagatacagcaagaagttcaagccggaaatagcaataagacccaaagtgagggatcaagaagggagaatgaactattactggacactagtagagccgggagacaaaataacattcgaagcaactggaaatctagtggtaccgagatatgcattcgcaatggaaagaaatgctggatctggtattatcatttcagatacaccagtccacgattgcaatacaacttgtcagacacccaagggtgctataaacaccagcctcccatttcagaatatacatccgatcacaattggaaaatgtccaaaatatgtaaaaagcacaaaattgagactggccacaggattgaggaatgtcccgtctattcaatctagaggcctatttggggccattgccggtttcattgaaggggggtggacagggatggtagatggatggtacggttatcaccatcaaaatgagcaggggtcaggatatgcagccgacctgaagagcacacagaatgccattgacgagattactaacaaagtaaattctgttattgaaaagatgaatacacagttcacagcagtaggtaaagagttcaaccacctggaaaaaagaatagagaatttaaataaaaaagttgatgatggtttcctggacatttggacttacaatgccgaactgttggttctattggaaaatgaaagaactttggactaccacgattcaaatgtgaagaacttatatgaaaaggtaagaagccagctaaaaaacaatgccaaggaaattggaaacggctgctttgaattttaccacaaatgcgataacacgtgcatggaaagtgtcaaaaatgggacttatgactacccaaaatactcagaggaagcaaaattaaacagagaagaaatagatggggtaaagctggaatcaacaaggatttaccagattttggcgatctattcaactgtcgccagttcattggtactggtagtctccctgggggcaatcagtttctggatgtgctctaatgggtctctacagtgtagaatatgtatttaacattaggatttcagaagcatgagaaaaacacccttgtttctactagcaaaagcagggtagataatcactcaatggcgtctcaaggcaccaaacgatcatatgaacaaatggagactggtggggagcgccaggatgccacagaaatcagagcatctgtcggaagaatgattggtggaatcgggagattctacatccaaatgtgcactgaactcaaactcagtgattatgatggacgactaatccagaatagcataacaatagagaggatggtgctttctgcttttgatgagagaagaaataaatacctagaagagcatcccagtgctgggaaggaccccaagaaaacaggaggacccatatatagaagagtagacggaaagtggatgagagaactcatcctttatgacaaagaagaaataaggagagtttggcgccaagcaaacaatggcgaagatgcaacagcaggtattactcatatcatgatttggcattccaacctgaatgatgccacatatcagagaacaagagcgcttgttcgcaccggaatggatcccagaatgtgctctctaatgcaaggttcaacacttcccagaaggtctggtgccgcaggtgctgcggtgaaaggagttggaacaatagcaatggagttaatcagaatgatcaaacgtggaatcaatgaccgaaatttctggaggggtgaaaatggacgaaggacaagggttgcttatgaaagaatgtgcaatatcctcaaaggaaaatttcaaacagctgcccagagggcaatgatggatcaagtaagagaaagtcgaaacccaggaaacgctgagattgaagacctcattttcctggcacggtcagcactcattctgaggggatcagttgcacataaatcctgcctgcctgcttgtgtgtatgggcttgcagtagcaagtgggcatgactttgaaagggaagggtactcactggtcgggatagacccattcaaattactccaaaacagccaagtggtcagcctgatgagaccaaatgaaaacccagctcacaagagtcaattggtgtggatggcatgccactctgctgcatttgaagatttaagagtatcaagtttcataagaggaaagaaagtgattccaagaggaaagctttccacaagaggggtccagattgcttcaaatgagaatgtggaaatcatggactccaataccctggaactgagaagcagatactgggccataaggaccaggagtggaggaaataccaatcaacaaaaggcatccgcaggccagatcagtgtgcagcctacattctcagtgcagcggaatctcccttttgaaagagcaaccgttatggcagcattcagcgggaacaatgaaggacggacatccgacatgcgaacagaagttataagaatgatggaaagtgcaaagccagaagatttgtccttccaggggcggggagtcttcgagctctcggacgaaaaggcaacgaacccgatcgtgccttcctttgacatgagtaatgaagggtcttatttcttcggagacaatgcagaggagtatgacagttgaggaaaaatacccttgtttctactagcaaaagcaggagtttaaaatgaatccaaaccaaaagataataaccattggttcggtctgtatgacaattggaatggctaacttaatattacaaattggaaacataatctcaacatggattagccactcaattcaacttgggaatcaaaatcagattgaaacatgcaatcaaagcgtcattacttatgaaaacaacacttgggtaaatcagacatatgttaacatcagcaacaccaactttgctgctggacagtcagtggtttccgtgaaattagcgggcaattcctctctctgccctgttagtggatgggctatatacagtaaagacaacagcgtaagaatcggttccaagggggatgtgtttgtcataagggaaccattcatatcatgctcccccttggaatgcagaaccttcttcttgactcaaggggccttgctaaatgacaaacattccaatggaaccattaaagacaggagcccatatcgaaccctaatgagctgtcctattggtgaagttccctctccatacaactcaagatttgagtcagtcgcttggtcagcaagtgcttgtcatgatggcatcaattggctaacaattggaatttctggcccagacaatggggcagtggctgtgttaaagtacaacggcataataacagacactatcaagagttggagaaacaatatattgagaacacaagagtctgaatgtgcatgtgtaaatggttcttgctttactgtaatgaccgatggaccaagtaatggacaggcctcatacaagatcttcagaatagaaaagggaaaaatagtcaaatcagtcgaaatgaatgcccctaattatcactatgaggaatgctcctgttatcctgattctagtgaaatcacatgtgtgtgcagggataactggcatggctcgaatcgaccgtgggtgtctttcaaccagaatctggaatatcagataggatacatatgcagtgggattttcggagacaatccacgccctaatgataagacaggcagttgtggtccagtatcgtctaatggagcaaatggagtaaaaggattttcattcaaatacggcaatggtgtttggatagggagaactaaaagcattagttcaagaaacggttttgagatgatttgggatccgaacggatggactgggacagacaataacttctcaataaagcaagatatcgtaggaataaatgagtggtcaggatatagcgggagttttgttcagcatccagaactaacagggctggattgtataagaccttgcttctgggttgaactaatcagagggcgacccaaagagaacacaatctggactagcgggagcagcatatccttttgtggtgtaaacagtgacactgtgggttggtcttggccagacggtgctgagttgccatttaccattgacaagtaatttgttcaaaaaactccttgtttctactagcaaaagcaggtagatatttaaagatgagtcttctaaccgaggtcgaaacgtacgttctttctatcatcccgtcaggccccctcaaagccgagatcgcgcagagactggaaagtgtctttgcaggaaagaacacagatcttgaggctctcatggaatggctaaagacaagaccaatcttgtcacctctgactaagggaattttaggatttgtgttcacgctcaccgtgcccagtgagcgaggactgcagcgtagacgctttgtccaaaatgccctaaatgggaatggggacccgaacaacatggatagagcagttaaactatacaagaagctcaaaagagaaataacgttccatggggccaaggaggtgtcactaagctattcaactggtgcacttgccagttgcatgggcctcatatacaacaggatgggaacagtgaccacagaagctgcttttggtctagtgtgtgccacttgtgaacagattgctgattcacagcatcggtctcacagacagatggctactaccaccaatccactaatcaggcatgaaaacagaatggtgctggctagcactacggcaaaggctatggaacagatggctggatcgagtgaacaggcagcggaggccatggaggttgctaatcagactaggcagatggtacatgcaatgagaactattgggactcatcctagctccagtgctggtctgaaagatgaccttcttgaaaatttgcaggcctaccagaagcgaatgggagtgcagatgcagcgattcaagtgatcctctcgtcattgcagcaaatatcattgggatcttgcacctgatattgtggattactgatcgtctttttttcaaatgtatttatcgtcgctttaaatacggtttgaaaagagggccttctacggaaggagtgcctgagtccatgagggaagaatatcaacaggaacagcagagtgctgtggatgttgacgatggtcattttgtcaacatagagctggagtaaaaaactaccttgtttctactagcaaaagcagggtgacaaaaacataatggactccaacaccatgtcaagctttcaggtagactgtttcctttggcatatccgcaagcgatttgcagacaatggattgggtgatgccccattccttgatcggctccgccgagatcaaaagtccttaaaaggaagaggcaacacccttggcctcgatatcgaaacagccactcttgttgggaaacaaatcgtggaatggatcttgaaagaggaatccagcgagacacttagaatgacaattgcatctgtacctacttcgcgctacctttctgacatgaccctcgaggaaatgtcacgagactggttcatgctcatgcctaggcaaaagataataggccctctttgcgtgcgattggaccaggcgatcatggaaaagtagatcttgattaattaagagggagcaatagttggagaaatttcaccattaccttctcttccaggacatacttatgaggatgtcaaaaatgcagttggggtcctcatcggaggacttgaatggaatggtaacacggttcgagtctctgaaaatatacagagattcgcttggagaaactgtgatgagaatgggagaccttcactacctccagagcagaaatgaaaagtggcgagagcaattgggacagaaatttgaggaaataaggtggttaattgaagaaatgcggcacagattgaaagcgacagagaatagtttcgaacaaataacatttatgcaagccttacaactattgcttgaagtagaacaagagataagagctttctcgtttcagcttatttaatgataaaaaacacccttgtttctact

SEQ ID NO: 4 - protein, 3591 aa, synthetic construct
  source 1..3591: note = VSV HA
MSVTVKRIIDNTVIVPKLPANEDPVEYPADYFRKSKEIPLYINTTKSLSDLRGYVYQGLKSGNVSIIHVNSYLYGALKDIRGKLDKDWSSFGINIGKAGDTIGIFDLVSLKALDGVLPDGVSDASRTSADDKWLPLYLLGLYRVGRTQMPEYRKKLMDGLTNQCKMINEQFEPLVPEGRDIFDVWGNDSNYTKIVAAVDMFFHMFKKHECASFRYGTIVSRFKDCAALATFGHLCKITGMSTEDVTTWILNREVADEMVQMMLPGQEIDKADSYMPYLIDFGLSSKSPYSSVKNPAFHFWGQLTALLLRSTRARNARQPDDIEYTSLTTAGLLYAYAVGSSADLAQQFCVGDNKYTPDDSTGGLTTNAPPQGRDVVEWLGWFEDQNRKPTPDMMQYAKRAVMSLQGLREKTIGKYAKSEFDKMDNLTKVREYLKSYSRLDQAVGEIDEIEAQRAEKSNYELFQEDGVEEHTKPSYFQAADDSDTESEPEIEDNQGLYAQDPEAEQVEGFIQGPLDDYADEEVDVVFTSDWKPPELESDEHGKTLRLTSPEGLSGEQKSQWLSTIKAVVQSAKYWNLAECTFEASGEGVIMKERQITPDVYKVTPVMNTHPSQSEAVSDVWSLSKTSMTFQPKKASLQPLTISLDELFSSRGEFISVGGDGRMSHKEAILLGLRYKKLYNQARVKYSLMSSLKKILGLKGKGKKSKKLGIAPPPYEEDTSMEYAPSAPIDKSYFGVDEMDTYDPNQLRYEKFFFTVKMTVRSNRPFRTYSDVAAAVSHWDHMYIGMAGKRPFYKILAFLGSSNLKATPAVLADQGQPEYHTHCEGRAYLPHRMGKTPPMLNVPEHFRRPFNIGLYKGTIELTMTIYDDESLEAAPMIWDHFNSSKFSDFREKALMFGLIVEKKASGAWVLDSISHFKMKAILVVLLYTFTTANADTLCIGYHANNSTDTVDTVLEKNVTVTHSVNLLEDKHNGKLCKLRGVAPLHLGKCNIAGWILGNPECESLSTASSWSYIVETSSSDNGTCYPGDFIDYEELREQLSSVSSFERFEIFPKTSSWPNHDSNKGVTAACPHAGAKSFYKNLIWLVKKGNSYPKLSKSYINDKGKEVLVLWGIHHPSTSADQQSLYQNADAYVFVGSSRYSKKFKPEIAIRPKVRDQEGRMNYYWTLVEPGDKITFEATGNLVVPRYAFAMERNAGSGIIISDTPVHDCNTTCQTPKGAINTSLPFQNIHPITIGKCPKYVKSTKLRLATGLRNVPSIQSRGLFGAIAGFIEGGWTGMVDGWYGYHHQNEQGSGYAADLKSTQNAIDEITNKVNSVIEKMNTQFTAVGKEFNHLEKRIENLNKKVDDGFLDIWTYNAELLVLLENERTLDYHDSNVKNLYEKVRSQLKNNAKEIGNGCFEFYHKCDNTCMESVKNGTYDYPKYSEEAKLNREEIDGVKLESTRIYQILAIYSTVASSLVLVVSLGAISFWMCSNGSLQCRICIMEVHDFETDEFNDFNEDDYATREFLNPDERMTYLNHADYNLNSPLISDDIDNLIRKFNSLPIPSMWDSKNWDGVLEMLTSCQANPISTSQMHKWMGSWLMSDNHDASQGYSFLHEVDKEAEITFDVVETFIRGWGNKPIEYIKKERWTDSFKILAYLCQKFLDLHKLTLILNAVSEVELLNLARTFKGKVRRSSHGTNICRIRVPSLGPTFISEGWAYFKKLDILMDRNFLLMVKDVIIGRMQTVLSMVCRIDNLFSEQDIFSLLNIYRIGDKIVERQGNFSYDLIKMVEPICNLKLMKLARESRPLVPQFPHFENHIKTSVDEGAKIDRGIRFLHDQIMSVKTVDLTLVIYGSFRHWGHPFIDYYTGLEKLHSQVTMKKDIDVSYAKALASDLARIVLFQQFNDHKKWFVNGDLLPHDHPFKSHVKENTWPTAAQVQDFGDKWHELPLIKCFEIPDLLDPSIIYSDKSHSMNRSEVLKHVRMNPNTPIPSKKVLQTMLDTKATNWKEFLKEIDEKGLDDDDLIIGLKGKERELKLAGRFFSLMSWKLREYFVITEYLIKTHFVPMFKGLTMADDLTAVIKKMLDSSSGQGLKSYEAICIANHIDYEKWNNHQRKLSNGPVFRVMGQFLGYPSLIERTHEFFEKSLIYYNGRPDLMRVHNNTLINSTSQRVCWQGQEGGLEGLRQKGWTILNLLVIQREAKIRNTAVKVLAQGDNQVICTQYKTKKSRNVVELQGALNQMVSNNEKIMTAIKIGTGKLGLLINDDETMQSADYLNYGKIPIFRGVIRGLETKRWSRVTCVTNDQIPTCANIMSSVSTNALTVAHFAENPINAMIQYNYFGTFARLLLMMHDPALRQSLYEVQDKIPGLHSSTFKYAMLYLDPSIGGVSGMSLSRFLIRAFPDPVTESLSFWRFIHVHARSEHLKEMSAVFGNPEIAKFRITHIDKLVEDPTSLNIAMGMSPANLLKTEVKKCLIESRQTIRNQVIKDATIYLYHEEDRLRSFLWSINPLFPRFLSEFKSGTFLGVADGLISLFQNSRTIRNSFKKKYHRELDDLIVRSEVSSLTHLGKLHLRRGSCKMWTCSATHADTLRYKSWGRTVIGTTVPHPLEMLGPQHRKETPCAPCNTSGFNYVSVHCPDGIHDVFSSRGPLPAYLGSKTSESTSILQPWERESKVPLIKRATRLRDAISWFVEPDSKLAMTILSNIHSLTGEEWTKRQHGFKRTGSALHRFSTSRMSHGGFASQSTAALTRLMATTDTMRDLGDQNFDFLFQATLLYAQITTTVARDGWITSCTDHYHIACKSCLRPIEEITLDSSMDYTPPDVSHVLKTWRNGEGSWGQEIKQIYPLEGNWKNLAPAEQSYQVGRCIGFLYGDLAYRKSTHAEDSSLFPLSIQGRIRGRGFLKGLLDGLMRASCCQVIHRRSLAHLKRPANAVYGGLIYLIDKLSVSPPFLSLTRSGPIRDELETIPHKIPTSYPTSNRDMGVIVRNYFKYQCRLIEKGKYRSHYSQLWLFSDVLSIDFIGPFSISTTLLQILYKPFLSGKDKNELRELANLSSLLRSGEGWEDIHVKFFTKDILLCPEEIRHACKFGIAKDNNKDMSYPPWGRESRGTITTIPVYYTTTPYPKMLEMPPRIQNPLLSGIRLGQLPTGAHYKIRSILHGMGIHYRDFLSCGDGSGGMTAALLRENVHSRGIFNSLLELSGSVMRGASPEPPSALETLGGDKSRCVNGETCWEYPSDLCDPRTWDYFLRLKAGLGLQIDLIVMDMEVRDSSTSLKIETNVRNYVHRILDEQGVLIYKTYGTYICESEKNAVTILGPMFKTVDLVQTEFSSSQTSEVYMVCKGLKKLIDEPNPDWSSINESWKNLYAFQSSEQEFARAKKVSTYFTLTGIPSQFIPDPFVNIETMLQIFGVPTGVSHAAALKSSDRPADLLTISLFYMAIISYYNINHIRVGPIPPNPPSDGIAQNVGIAITGISFWLSLMEKDIPLYQQCLAVIQQSFPIRWEAVSVKGGYKQKWSTRGDGLPKDTRTSDSLAPIGNWIRSLELVRNQVRLNPFNEILFNQLCRTVDNHLKWSNLRRNTGMIEWINRRISKEDRSILMLKSDLHEENSWRD

SEQ ID NO: 5 - protein, 4593 aa, synthetic construct
  source 1..4593: note = NS1(1-126)
MERIKELRDLMSQSRTREILTKTTVDHMAIIKKYTSGRQEKNPALRMKWMMAMRYPITADKRIMDMIPERNEQGQTLWSKTNDAGSDRVMVSPLAVTWWNRNGPTTSTVHYPKVYKTYFEKVERLKHGTFGPVHFRNQVKIRRRVDTNPGHADLSAKEAQDVIMEVVFPNEVGARILTSESQLAITKEKKEELQDCKIAPLMVAYMLERELVRKTRFLPVAGGTGSVYIEVLHLTQGTCWEQMYTPGGEVRNDDVDQSLIIAARNIVRRAAVSADPLASLLEMCHSTQIGGVRMVDILRQNPTEEQAVDICKAAIGLRISSSFSFGGFTFKRTSGSSVKKEEEVLTGNLQTLKIRVHEGYEEFTMVGRRATAILRKATRRLIQLIVSGRDEQSIAEAIIVAMVFSQEDCMIKAVRGDLNFVNRANQRLNPMHQLLRHFQKDAKVLFQNWGIESIDNVMGMIGILPDMTPSTEMSLRGIRVSKMGVDEYSSTERVVVSIDRFLRVRDQRGNVLLSPEEVSETQGTERLTITYSSSMMWEINGPESVLVNTYQWIIRNWEIVKIQWSQDPTMLYNKMEFEPFQSLVPKATRSRYSGFVRTLFQQMRDVLGTFDTVQIIKLLPFAAAPPEQSRMQFSSLTVNVRGSGLRILVRGNSPVFNYNKATKRLTVLGKDAGALTEDPDEGTSGVESAVLRGFLILGKEDKRYGPALSINELSNLAKGEKANVLIGQGDVVLVMKRKRDSSILTDSQTATKRIRMAINMDVNPTLLFLKIPAQNAISTTFPYTGDPPYSHGTGTGYTMDTVNRTHQYSEKGKWTTNTETGAPQLNPIDGPLPEDNEPSGYAQTDCVLEAMAFLEESHPGIFENSCLETMEVVQQTRVDKLTQGRQTYDWTLNRNQPAATALANTIEVFRSNGLTANESGRLIDFLKDVMESMNKEEIEITTHFQRKRRVRDNMTKKMVTQRTIGKKKQRLNKRGYLIRALTLNTMTKDAERGKLKRRAIATPGMQIRGFVYFVETLARSICEKLEQSGLPVGGNEKKAKLANVVRKMMTNSQDTEISFTITGDNTKWNENQNPRVFLAMITYITRNQPEWFRNILSMAPIMFSNKMARLGKGYMFESKRMKIRTQIPAEMLASIDLKYFNESTKKKIEKIRPLLIDGTASLSPGMMMGMFNMLSTVLGVSILNLGQKKYTKTIYWWDGLQSSDDFALIVNAPNHEGIQAGVDRFYRTCKLVGINMSKKKSYINKTGTFEFTSFFYRYGFVANFSMELPSFGVSGVNESADMSIGVTVIKNNMINNDLGPATAQMALQLFIKDYRYTYRCHRGDTQIQTRRSFELKKLWDQTQSKVGLLVSDGGPNLYNIRNLHIPEVCLKWELMDDDYRGRLCNPLNPFVSHKEIDSVNNAVVMPAHGPAKSMEYDAVATTHSWIPKRNRSILNTSQRGILEDEQMYQKCCNLFEKFFPSSSYRRPVGISSMVEAMVSRARIDARVDFESGRIKKEEFSEIMKICSTIEELRRQKMEDFVRQCFNPMIVELAEKAMKEYGEDPKIETNKFAAICTHLEVCFMYSDFHFIDERGESIIVESGDPNALLKHRFEIIEGRDRIMAWTVVNSICNTTGVEKPKFLPDLYDYKENRFIEIGVTRREVHIYYLEKANKIKSEKTHIHIFSFTGEEMATKADYTLDEESRARIKTRLFTIRQEMASRSLWDSFRQSERGEETIEEKFEITGTMRKLADQSLPPNFSSLENFRAYVDGFEPNGCIEGKLSQMSKEVNAKIEPFLRTTPRPLRLPDGPLCHQRSKFLLMDALKLSIEDPSHEGEGIPLYDAIKCMKTFFGWKEPNIVKPHEKGINPNYLMAWKQVLAELQDIENEEKIPRTKNMKRTSQLKWALGENMAPEKVDFDDCKDVGDLKQYDSDEPEPRSLASWVQNEFNKACELTDSSWIELDEIGEDVAPIEHIASMRRNYFTAEVSHCRATEYIMKGVYINTALLNASCAAMDDFQLIPMISKCRTKEGRRKTNLYGFIIKGRSHLRNDTDVVNFVSMEFSLTDPRLEPHKWEKYCVLEIGDMLLRTAIGQVSRPMFLYVRTNGTSKIKMKWGMELRRCLLQSLQQIESMIEAESSVKEKDMTKEFFENKSETWPIGESPRGVEEGSIGKVCRTLLAKSVFNSLYASPQLEGFSAESRKLLLIVQALRDNLEPGTFDLGGLYEAIEECLINDPWVLLNASWFNSFLTHALKMEDFVRQCFNPMIVELAEKAMKEYGEDPKIETNKFAAICTHLEVCFMYSDFHFIDERGESIIVESGDPNALLKHRFEIIEGRDRIMAWTVVNSICNTTGVEKPKFLPDLYDYKENRFIEIGVTRREVHIYYLEKANKIKSEKTHIHIFSFTGEEMATKADYTLDEESRARIKTRLFTIRQEMASRSLWDSFVSPKEAKRQLKKNLRLQELCASLPTKVSHRTSPALKTLEPMMKAILVVLLYTFTTANADTLCIGYHANNSTDTVDTVLEKNVTVTHSVNLLEDKHNGKLCKLRGVAPLHLGKCNIAGWILGNPECESLSTASSWSYIVETSSSDNGTCYPGDFIDYEELREQLSSVSSFERFEIFPKTSSWPNHDSNKGVTAACPHAGAKSFYKNLIWLVKKGNSYPKLSKSYINDKGKEVLVLWGIHHPSTSADQQSLYQNADAYVFVGSSRYSKKFKPEIAIRPKVRDQEGRMNYYWTLVEPGDKITFEATGNLVVPRYAFAMERNAGSGIIISDTPVHDCNTTCQTPKGAINTSLPFQNIHPITIGKCPKYVKSTKLRLATGLRNVPSIQSRGLFGAIAGFIEGGWTGMVDGWYGYHHQNEQGSGYAADLKSTQNAIDEITNKVNSVIEKMNTQFTAVGKEFNHLEKRIENLNKKVDDGFLDIWTYNAELLVLLENERTLDYHDSNVKNLYEKVRSQLKNNAKEIGNGCFEFYHKCDNTCMESVKNGTYDYPKYSEEAKLNREEIDGVKLESTRIYQILAIYSTVASSLVLVVSLGAISFWMCSNGSLQCRICIMASQGTKRSYEQMETGGERQDATEIRASVGRMIGGIGRFYIQMCTELKLSDYDGRLIQNSITIERMVLSAFDERRNKYLEEHPSAGKDPKKTGGPIYRRVDGKWMRELILYDKEEIRRVWRQANNGEDATAGITHIMIWHSNLNDATYQRTRALVRTGMDPRMCSLMQGSTLPRRSGAAGAAVKGVGTIAMELIRMIKRGINDRNFWRGENGRRTRVAYERMCNILKGKFQTAAQRAMMDQVRESRNPGNAEIEDLIFLARSALILRGSVAHKSCLPACVYGLAVASGHDFEREGYSLVGIDPFKLLQNSQVVSLMRPNENPAHKSQLVWMACHSAAFEDLRVSSFIRGKKVIPRGKLSTRGVQIASNENVEIMDSNTLELRSRYWAIRTRSGGNTNQQKASAGQISVQPTFSVQRNLPFERATVMAAFSGNNEGRTSDMRTEVIRMMESAKPEDLSFQGRGVFELSDEKATNPIVPSFDMSNEGSYFFGDNAEEYDSMNPNQKIITIGSVCMTIGMANLILQIGNIISTWISHSIQLGNQNQIETCNQSVITYENNTWVNQTYVNISNTNFAAGQSVVSVKLAGNSSLCPVSGWAIYSKDNSVRIGSKGDVFVIREPFISCSPLECRTFFLTQGALLNDKHSNGTIKDRSPYRTLMSCPIGEVPSPYNSRFESVAWSASACHDGINWLTIGISGPDNGAVAVLKYNGIITDTIKSWRNNILRTQESECACVNGSCFTVMTDGPSNGQASYKIFRIEKGKIVKSVEMNAPNYHYEECSCYPDSSEITCVCRDNWHGSNRPWVSFNQNLEYQIGYICSGIFGDNPRPNDKTGSCGPVSSNGANGVKGFSFKYGNGVWIGRTKSISSRNGFEMIWDPNGWTGTDNNFSIKQDIVGINEWSGYSGSFVQHPELTGLDCIRPCFWVELIRGRPKENTIWTSGSSISFCGVNSDTVGWSWPDGAELPFTIDKMSLLTEVETYVLSIIPSGPLKAEIAQRLESVFAGKNTDLEALMEWLKTRPILSPLTKGILGFVFTLTVPSERGLQRRRFVQNALNGNGDPNNMDRAVKLYKKLKREITFHGAKEVSLSYSTGALASCMGLIYNRMGTVTTEAAFGLVCATCEQIADSQHRSHRQMATTTNPLIRHENRMVLASTTAKAMEQMAGSSEQAAEAMEVANQTRQMVHAMRTIGTHPSSSAGLKDDLLENLQAYQKRMGVQMQRFKMSLLTEVETPTRSEWECRCSDSSDPLVIAANIIGILHLILWITDRLFFKCIYRRFKYGLKRGPSTEGVPESMREEYQQEQQSAVDVDDGHFVNIELEMDSNTMSSFQVDCFLWHIRKRFADNGLGDAPFLDRLRRDQKSLKGRGNTLGLDIETATLVGKQIVEWILKEESSETLRMTIASVPTSRYLSDMTLEEMSRDWFMLMPRQKIIGPLCVRLDQAIMEKMDSNTMSSFQDILMRMSKMQLGSSSEDLNGMVTRFESLKIYRDSLGETVMRMGDLHYLQSRNEKWREQLGQKFEEIRWLIEEMRHRLKATENSFEQITFMQALQLLLEVEQEIRAFSFQLI

SEQ ID NO: 6 - protein, 4361 aa, synthetic construct
  source 1..4361: note = NS1(1-126)-deltaPAX
MERIKELRDLMSQSRTREILTKTTVDHMAIIKKYTSGRQEKNPALRMKWMMAMRYPITADKRIMDMIPERNEQGQTLWSKTNDAGSDRVMVSPLAVTWWNRNGPTTSTVHYPKVYKTYFEKVERLKHGTFGPVHFRNQVKIRRRVDTNPGHADLSAKEAQDVIMEVVFPNEVGARILTSESQLAITKEKKEELQDCKIAPLMVAYMLERELVRKTRFLPVAGGTGSVYIEVLHLTQGTCWEQMYTPGGEVRNDDVDQSLIIAARNIVRRAAVSADPLASLLEMCHSTQIGGVRMVDILRQNPTEEQAVDICKAAIGLRISSSFSFGGFTFKRTSGSSVKKEEEVLTGNLQTLKIRVHEGYEEFTMVGRRATAILRKATRRLIQLIVSGRDEQSIAEAIIVAMVFSQEDCMIKAVRGDLNFVNRANQRLNPMHQLLRHFQKDAKVLFQNWGIESIDNVMGMIGILPDMTPSTEMSLRGIRVSKMGVDEYSSTERVVVSIDRFLRVRDQRGNVLLSPEEVSETQGTERLTITYSSSMMWEINGPESVLVNTYQWIIRNWEIVKIQWSQDPTMLYNKMEFEPFQSLVPKATRSRYSGFVRTLFQQMRDVLGTFDTVQIIKLLPFAAAPPEQSRMQFSSLTVNVRGSGLRILVRGNSPVFNYNKATKRLTVLGKDAGALTEDPDEGTSGVESAVLRGFLILGKEDKRYGPALSINELSNLAKGEKANVLIGQGDVVLVMKRKRDSSILTDSQTATKRIRMAINMDVNPTLLFLKIPAQNAISTTFPYTGDPPYSHGTGTGYTMDTVNRTHQYSEKGKWTTNTETGAPQLNPIDGPLPEDNEPSGYAQTDCVLEAMAFLEESHPGIFENSCLETMEVVQQTRVDKLTQGRQTYDWTLNRNQPAATALANTIEVFRSNGLTANESGRLIDFLKDVMESMNKEEIEITTHFQRKRRVRDNMTKKMVTQRTIGKKKQRLNKRGYLIRALTLNTMTKDAERGKLKRRAIATPGMQIRGFVYFVETLARSICEKLEQSGLPVGGNEKKAKLANVVRKMMTNSQDTEISFTITGDNTKWNENQNPRVFLAMITYITRNQPEWFRNILSMAPIMFSNKMARLGKGYMFESKRMKIRTQIPAEMLASIDLKYFNESTKKKIEKIRPLLIDGTASLSPGMMMGMFNMLSTVLGVSILNLGQKKYTKTIYWWDGLQSSDDFALIVNAPNHEGIQAGVDRFYRTCKLVGINMSKKKSYINKTGTFEFTSFFYRYGFVANFSMELPSFGVSGVNESADMSIGVTVIKNNMINNDLGPATAQMALQLFIKDYRYTYRCHRGDTQIQTRRSFELKKLWDQTQSKVGLLVSDGGPNLYNIRNLHIPEVCLKWELMDDDYRGRLCNPLNPFVSHKEIDSVNNAVVMPAHGPAKSMEYDAVATTHSWIPKRNRSILNTSQRGILEDEQMYQKCCNLFEKFFPSSSYRRPVGISSMVEAMVSRARIDARVDFESGRIKKEEFSEIMKICSTIEELRRQKMEDFVRQCFNPMIVELAEKAMKEYGEDPKIETNKFAAICTHLEVCFMYSDFHFIDERGESIIVESGDPNALLKHRFEIIEGRDRIMAWTVVNSICNTTGVEKPKFLPDLYDYKENRFIEIGVTRREVHIYYLEKANKIKSEKTHIHIFSFTGEEMATKADYTLDEESRARIKTRLFTIRQEMASRSLWDSFRQSERGEETIEEKFEITGTMRKLADQSLPPNFSSLENFRAYVDGFEPNGCIEGKLSQMSKEVNAKIEPFLRTTPRPLRLPDGPLCHQRSKFLLMDALKLSIEDPSHEGEGIPLYDAIKCMKTFFGWKEPNIVKPHEKGINPNYLMAWKQVLAELQDIENEEKIPRTKNMKRTSQLKWALGENMAPEKVDFDDCKDVGDLKQYDSDEPEPRSLASWVQNEFNKACELTDSSWIELDEIGEDVAPIEHIASMRRNYFTAEVSHCRATEYIMKGVYINTALLNASCAAMDDFQLIPMISKCRTKEGRRKTNLYGFIIKGRSHLRNDTDVVNFVSMEFSLTDPRLEPHKWEKYCVLEIGDMLLRTAIGQVSRPMFLYVRTNGTSKIKMKWGMELRRCLLQSLQQIESMIEAESSVKEKDMTKEFFENKSETWPIGESPRGVEEGSIGKVCRTLLAKSVFNSLYASPQLEGFSAESRKLLLIVQALRDNLEPGTFDLGGLYEAIEECLINDPWVLLNASWFNSFLTHALKMKAILVVLLYTFTTANADTLCIGYHANNSTDTVDTVLEKNVTVTHSVNLLEDKHNGKLCKLRGVAPLHLGKCNIAGWILGNPECESLSTASSWSYIVETSSSDNGTCYPGDFIDYEELREQLSSVSSFERFEIFPKTSSWPNHDSNKGVTAACPHAGAKSFYKNLIWLVKKGNSYPKLSKSYINDKGKEVLVLWGIHHPSTSADQQSLYQNADAYVFVGSSRYSKKFKPEIAIRPKVRDQEGRMNYYWTLVEPGDKITFEATGNLVVPRYAFAMERNAGSGIIISDTPVHDCNTTCQTPKGAINTSLPFQNIHPITIGKCPKYVKSTKLRLATGLRNVPSIQSRGLFGAIAGFIEGGWTGMVDGWYGYHHQNEQGSGYAADLKSTQNAIDEITNKVNSVIEKMNTQFTAVGKEFNHLEKRIENLNKKVDDGFLDIWTYNAELLVLLENERTLDYHDSNVKNLYEKVRSQLKNNAKEIGNGCFEFYHKCDNTCMESVKNGTYDYPKYSEEAKLNREEIDGVKLESTRIYQILAIYSTVASSLVLVVSLGAISFWMCSNGSLQCRICIMASQGTKRSYEQMETGGERQDATEIRASVGRMIGGIGRFYIQMCTELKLSDYDGRLIQNSITIERMVLSAFDERRNKYLEEHPSAGKDPKKTGGPIYRRVDGKWMRELILYDKEEIRRVWRQANNGEDATAGITHIMIWHSNLNDATYQRTRALVRTGMDPRMCSLMQGSTLPRRSGAAGAAVKGVGTIAMELIRMIKRGINDRNFWRGENGRRTRVAYERMCNILKGKFQTAAQRAMMDQVRESRNPGNAEIEDLIFLARSALILRGSVAHKSCLPACVYGLAVASGHDFEREGYSLVGIDPFKLLQNSQVVSLMRPNENPAHKSQLVWMACHSAAFEDLRVSSFIRGKKVIPRGKLSTRGVQIASNENVEIMDSNTLELRSRYWAIRTRSGGNTNQQKASAGQISVQPTFSVQRNLPFERATVMAAFSGNNEGRTSDMRTEVIRMMESAKPEDLSFQGRGVFELSDEKATNPIVPSFDMSNEGSYFFGDNAEEYDSMNPNQKIITIGSVCMTIGMANLILQIGNIISTWISHSIQLGNQNQIETCNQSVITYENNTWVNQTYVNISNTNFAAGQSVVSVKLAGNSSLCPVSGWAIYSKDNSVRIGSKGDVFVIREPFISCSPLECRTFFLTQGALLNDKHSNGTIKDRSPYRTLMSCPIGEVPSPYNSRFESVAWSASACHDGINWLTIGISGPDNGAVAVLKYNGIITDTIKSWRNNILRTQESECACVNGSCFTVMTDGPSNGQASYKIFRIEKGKIVKSVEMNAPNYHYEECSCYPDSSEITCVCRDNWHGSNRPWVSFNQNLEYQIGYICSGIFGDNPRPNDKTGSCGPVSSNGANGVKGFSFKYGNGVWIGRTKSISSRNGFEMIWDPNGWTGTDNNFSIKQDIVGINEWSGYSGSFVQHPELTGLDCIRPCFWVELIRGRPKENTIWTSGSSISFCGVNSDTVGWSWPDGAELPFTIDKMSLLTEVETYVLSIIPSGPLKAEIAQRLESVFAGKNTDLEALMEWLKTRPILSPLTKGILGFVFTLTVPSERGLQRRRFVQNALNGNGDPNNMDRAVKLYKKLKREITFHGAKEVSLSYSTGALASCMGLIYNRMGTVTTEAAFGLVCATCEQIADSQHRSHRQMATTTNPLIRHENRMVLASTTAKAMEQMAGSSEQAAEAMEVANQTRQMVHAMRTIGTHPSSSAGLKDDLLENLQAYQKRMGVQMQRFKMSLLTEVETPTRSEWECRCSDSSDPLVIAANIIGILHLILWITDRLFFKCIYRRFKYGLKRGPSTEGVPESMREEYQQEQQSAVDVDDGHFVNIELEMDSNTMSSFQVDCFLWHIRKRFADNGLGDAPFLDRLRRDQKSLKGRGNTLGLDIETATLVGKQIVEWILKEESSETLRMTIASVPTSRYLSDMTLEEMSRDWFMLMPRQKIIGPLCVRLDQAIMEKMDSNTMSSFQDILMRMSKMQLGSSSEDLNGMVTRFESLKIYRDSLGETVMRMGDLHYLQSRNEKWREQLGQKFEEIRWLIEEMRHRLKATENSFEQITFMQALQLLLEVEQEIRAFSFQLI